European Patent Application EP 4 559 472 A1, published May 28, 2025. Title: Complement modulator. Applicant: Universität Ulm. The sequence listing filed with the application follows.

SEQUENCE LISTING (12 sequences)

SEQ ID NO: 1 - protein, 127 aa, synthetic construct
AGGKCGPPPPIDNGDITSFPLSVYAPASSVEYQCQNLYQLEGNKRITCRNGQWSEPPKCLHPCVISREIMENYNIALRWTAKQKLYSRTGESVEFVCKRGYRLSSRSHTLRTTCWDGKLEYPTCAKR

SEQ ID NO: 2 - protein, 127 aa, synthetic construct
AGGKCGPPPPIDNGGITSFPLSVYAPASSVEYQCQNLYQLEGNKRITCRNGQWSEPPKCLHPCVISREIMENYNIALRWTAKQKLYSRTGESVEFVCKRGYRLSSRSHTLRTTCWDGKLEYPTCAKR

SEQ ID NO: 3 - protein, 250 aa, synthetic construct
AGNCGPPPTLSFAAPMDITLTETRFKTGTTLKYTCLPGYVRSHSTQTLTCNSDGEWVYNTFCIYKRCRHPGELRNGQVEIKTDLSFGSQIEFSCSEGFFLIGSTTSRCEVQDRGVGWSHPLPQCEIVKCKPPPDIRNGRHSGEENFYAYGFSVTYSCDPRFSLLGHASISCTVENETIGVWRPSPPTCEKITCRKPDVSHGEMVSGFGPIYNYKDTIVFKCQKGFVLRGSSVIHCDADSKWNPSPPACEP

SEQ ID NO: 4 - protein, 381 aa, synthetic construct
AGNCGPPPTLSFAAPMDITLTETRFKTGTTLKYTCLPGYVRSHSTQTLTCNSDGEWVYNTFCIYKRCRHPGELRNGQVEIKTDLSFGSQIEFSCSEGFFLIGSTTSRCEVQDRGVGWSHPLPQCEIVKCKPPPDIRNGRHSGEENFYAYGFSVTYSCDPRFSLLGHASISCTVENETIGVWRPSPPTCEKITCRKPDVSHGEMVSGFGPIYNYKDTIVFKCQKGFVLRGSSVIHCDADSKWNPSPPACEPGGGGGGGKCGPPPPIDNGGITSFPLSVYAPASSVEYQCQNLYQLEGNKRITCRNGQWSEPPKCLHPCVISREIMENYNIALRWTAKQKLYSRTGESVEFVCKRGYRLSSRSHTLRTTCWDGKLEYPTCAKR

SEQ ID NO: 5 - protein, 381 aa, synthetic construct
AGNCGPPPTLSFAAPMDITLTETRFKTGTTLKYTCLPGYVRSHSTQTLTCNSDGEWVYNTFCIYKRCRHPGELRNGQVEIKTDLSFGSQIEFSCSEGFFLIGSTTSRCEVQDRGVGWSHPLPQCEIVKCKPPPDIRNGRHSGEENFYAYGFSVTYSCDPRFSLLGHASISCTVENETIGVWRPSPPTCEKITCRKPDVSHGEMVSGFGPIYNYKDTIVFKCQKGFVLRGSSVIHCDADSKWNPSPPACEPGGGGGGGKCGPPPPIDNGDITSFPLSVYAPASSVEYQCQNLYQLEGNKRITCRNGQWSEPPKCLHPCVISREIMENYNIALRWTAKQKLYSRTGESVEFVCKRGYRLSSRSHTLRTTCWDGKLEYPTCAKR

SEQ ID NO: 6 - protein, 504 aa, synthetic construct
AGNCGPPPTLSFAAPMDITLTETRFKTGTTLKYTCLPGYVRSHSTQTLTCNSDGEWVYNTFCIYKRCRHPGELRNGQVEIKTDLSFGSQIEFSCSEGFFLIGSTTSRCEVQDRGVGWSHPLPQCEIVKCKPPPDIRNGRHSGEENFYAYGFSVTYSCDPRFSLLGHASISCTVENETIGVWRPSPPTCEKITCRKPDVSHGEMVSGFGPIYNYKDTIVFKCQKGFVLRGSSVIHCDADSKWNPSPPACEPGGGGGGNCGPPPTLSFAAPMDITLTETRFKTGTTLKYTCLPGYVRSHSTQTLTCNSDGEWVYNTFCIYKRCRHPGELRNGQVEIKTDLSFGSQIEFSCSEGFFLIGSTTSRCEVQDRGVGWSHPLPQCEIVKCKPPPDIRNGRHSGEENFYAYGFSVTYSCDPRFSLLGHASISCTVENETIGVWRPSPPTCEKITCRKPDVSHGEMVSGFGPIYNYKDTIVFKCQKGFVLRGSSVIHCDADSKWNPSPPACEP

SEQ ID NO: 7 - protein, 604 aa, synthetic construct
AGCPAPELLGGPSVFLFPPKPKDTLMISRTPEVTCVVVDVSHEDPEVKFNWYVDGVEVHNAKTKPREEQYQSTYRVVSVLTVLHQDWLNGKEYKCKVSNKALPAPIEKTISKAKGQPREPQVYTLPPSREEMTKNQVSLTCLVKGFYPSDIAVEWESNGQPENNYKTTPPVLDSDGSFFLYSKLTVDKSRWQQGNVFSCSVMHEALHNHYTQKSLSLSPGGGGGGNCGPPPTLSFAAPMDITLTETRFKTGTTLKYTCLPGYVRSHSTQTLTCNSDGEWVYNTFCIYKRCRHPGELRNGQVEIKTDLSFGSQIEFSCSEGFFLIGSTTSRCEVQDRGVGWSHPLPQCEIVKCKPPPDIRNGRHSGEENFYAYGFSVTYSCDPRFSLLGHASISCTVENETIGVWRPSPPTCEKITCRKPDVSHGEMVSGFGPIYNYKDTIVFKCQKGFVLRGSSVIHCDADSKWNPSPPACEPGGGGGGGKCGPPPPIDNGGITSFPLSVYAPASSVEYQCQNLYQLEGNKRITCRNGQWSEPPKCLHPCVISREIMENYNIALRWTAKQKLYSRTGESVEFVCKRGYRLSSRSHTLRTTCWDGKLEYPTCAKR

SEQ ID NO: 8 - protein, 251 aa, synthetic construct
DCGLPPDVPNAQPALEGRTSFPEDTVITYKCEESFVKIPGEKDSVICLKGSQWSDIEEFCNRSCEVPTRLNSASLKQPYITQNYFPVGTVVEYECRPGYRREPSLSPKLTCLQNLKWSTAVEFCKKKSCPNPGEIRNGQIDVPGGILFGATISFSCNTGYKLFGSTSSFCLISGSSVQWSDPLPECREIYCPAPPQIDNGIIQGERDHYGYRQSVTYACNKGFTMIGEHSIYCTVNNDEGEWSGPPPECRG

SEQ ID NO: 9 - protein, 251 aa, synthetic construct
CEEPPTFEAMELIGKPKPYYEIGERVDYKCKKGYFYIPPLATHTICDRNHTWLPVSDDACYRETCPYIRDPLNGQAVPANGTYEFGYQMHFICNEGYYLIGEEILYCELKGSVAIWSGKPPICEKVLCTPPPKIKNGKHTFSEVEVFEYLDAVTYSCDPAPGPDPFSLIGESTIYCGDNSVWSRAAPECKVVKCRFPVVENGKQISGFGKKFYYKATVMFECDKGFYLDGSDTIVCDSNSTWDPPVPKCLK

SEQ ID NO: 10 - protein, 193 aa, synthetic construct
QCNAPEWLPFARPTNLTDEFEFPIGTYLNYECRPGYSGRPFSIICLKNSVWTGAKDRCRRKSCRNPPDPVNGMVHVIKGIQFGSQIKYSCTKGYRLIGSSSATCIISGDTVIWDNETPICDRIPCGLPPTITNGDFISTNRENFHYGSVVTYRCNPGSGGRKVFELVGEPSIYCTSNDDQVGIWSGPAPQCII

SEQ ID NO: 11 - protein, 194 aa, synthetic construct
GHCQAPDHFLFAKLKTQTNASDFPIGTSLKYECRPEYYGRPFSITCLDNLVWSSPKDVCKRKSCKTPPDPVNGMVHVITDIQVGSRINYSCTTGHRLIGHSSAECILSGNAAHWSTKPPICQRIPCGLPPTIANGDFISTNRENFHYGSVVTYRCNPGSGGRKVFELVGEPSIYCTSNDDQVGIWSGPAPQCII

SEQ ID NO: 12 - protein, 194 aa, synthetic construct
GHCQAPDHFLFAKLKTQTNASDFPIGTSLKYECRPEYYGRPFSITCLDNLVWSSPKDVCKRKSCKTPPDPVNGMVHVITDIQVGSRINYSCTTGHRLIGHSSAECILSGNTAHWSTKPPICQRIPCGLPPTIANGDFISTNRENFHYGSVVTYRCNLGSRGRKVFELVGEPSIYCTSNDDQVGIWSGPAPQCII